European Patent Application EP 4 242 660 A1, published September 13, 2023. Title: Reagent for measuring L-biotin, method for measuring samples containing L-biotin, method for determining the number of labels in L-biotin-labeled substance and method for producing optical isomeric avidins-immobilized solid phase. Applicant: SYSMEX CORPORATION. The sequence listing filed with the application follows.

SEQUENCE LISTING (33 sequences)

SEQ ID NO: 1 - protein, 159 aa, Streptomyces avidinii
  REGION 1..159: note = 90% or more of the amino acid residues other than glycine in the core sequence are D-amino acid residues
DPSKDSKAQVSAAEAGITGTWYNQLGSTFIVTAGADGALTGTYESAVGNAESRYVLTGRYDSAPATDGSGTALGWTVAWKNNYRNAHSATTWSGQYVGGAEARINTQWLLTSGTTEANAWKSTLVGHDTFTKVKPSAASIDAAKKAGVNNGNPLDAVQQ

SEQ ID NO: 2 - protein, 128 aa, Gallus gallus
ARKCSLTGKWTNDLGSNMTIGAVNSRGEFTGTYITAVTATSNEIKESPLHGTQNTINKRTQPTFGFTVNWKFSESTTVFTGQCFIDRNGKEVLKTMWLLRSSVNDIGDDWKATRVGINIFTRLRTQKE

SEQ ID NO: 3 - protein, 143 aa, Pleurotus cornucopiae
MKDVQSLLTGTWYNELGSTMNLTANKDGSLTGTYHSNVGEVPPTYHLSGRYNLQPPSGQGVTLGWAVSFENTSANVHSVSTWSGQYFSEPAEVILTQWLLSRSSEREDLWQSTHVGHDEFSKTKPTKEKIAQAQLLRRGLKFE

SEQ ID NO: 4 - protein, 141 aa, Pleurotus cornucopiae
MSDVQSSLTGTWYNELNSKMELTANKDGTLTGKYLSKVGDVYVPYPLSGRYNLQPPAGQGVALGWAVSWENSKIHSATTWSGQFFSESSPVILTQWLLSSSTARGDVWESTLVGNDSFTKTAPTEQQIAHAQLHCRAPRLK

SEQ ID NO: 5 - protein, 159 aa, synthetic construct
  REGION 1..159: note = Comprising modified amino acid sequence.
DPSKDSKAQVSAAEAGITGTWYNQLGSTFIVTAGADGALTGTYEAAVGNAESRYVLTGRYDSAPATDGSGTALGWTVAWKNNYRNAHSAATWSGQYVGGAEARINTQWLLTSGTTEANAWKSTLVGHATFTKVKPSAASIDAAKKAGVNNGNPLDAVQQ

SEQ ID NO: 6 - protein, 159 aa, synthetic construct
  REGION 1..159: note = Comprising modified amino acid sequence.
DPSKDSKAQVSAAEAGITGTWYNQLGSTFIVTAGADGALTGTYESAVGNAESRYTLTGRYDSAPARDGSGTALGWTVAWKNNYRNAHSATTWSGQYVGGAEARINTQWTLTSGTTEANAWKSTLRGHDTFTKVKPSAASIDAAKKAGVNNGNPLDAVQQ

SEQ ID NO: 7 - protein, 114 aa, synthetic construct
  REGION 1..114: note = Comprising modified amino acid sequence.
AEAGITGTWYNQSGSTFTVTAGADGNLTGQYENRAQGTGCQNSPYTLTGRYNGTKLEWRVEWNNSTENCHSRTEWRGQYQGGAEARINTQWNLTYEGGSGPATEQGQDTFTKVK

SEQ ID NO: 8 - protein, 151 aa, synthetic construct
  REGION 1..151: note = Comprising modified amino acid sequence.
DPSKDSKAQVSAAEAGITGTWYNQLGSTFIVTAGADGALTGTYESAVGNAESRYVLTGRYDSAPATDGSGTALGWTVAWKNNYRNAHSATTWSGQYVGGAEARINTQWLLTSKSTLVGDDTFTKVKPSAASIDAAKKAGVNNGNPLDAVQQ

SEQ ID NO: 9 - protein, 273 aa, synthetic construct
  REGION 1..273: note = Comprising modified amino acid sequence.
EANAKKSTLVGHDTFTKVKPSAASGGGSAEAGITGTWYNQLGSTFIVTAGADGALTGTYESAVGNAESRYVLTGRYDSAPATDGSGTALGWTVAWKNNYRNAHSATTWSGQYVGGAEARINTQWLLTSGTGSGTALGWTVAWKNNYRNAHSATTWSGQYVGGAEARINTQWLLTSGTTEANAWKSTLVGHDTFTKVKPSAASGGGSAEVGITGTWYNQLGSTFIVTAGADGALTGTYESAVGNAESRYVLTGRYDSAPATDGAAALEHHHHHH

SEQ ID NO: 10 - protein, 115 aa, Streptomyces avidinii
  REGION 1..115: note = 90% or more of the amino acid residues other than glycine in the core sequence are D-amino acid residues
GTWYNQLGSTFIVTAGADGALTGTYESAVGNAESRYVLTGRYDSAPATDGSGTALGWTVAWKNNYRNAHSATTWSGQYVGGAEARINTQWLLTSGTTEANAWKSTLVGHDTFTKV

SEQ ID NO: 11 - protein, 121 aa, Streptomyces avidinii
  REGION 1..121: note = 90% or more of the amino acid residues other than glycine in the partial sequence are D-amino acid residues
AEAGITGTWYNQLGSTFIVTAGADGALTGTYESAVGNAESRYVLTGRYDSAPATDGSGTALGWTVAWKNNYRNAHSATTWSGQYVGGAEARINTQWLLTSGTTEANAWKSTLVGHDTFTKV

SEQ ID NO: 12 - protein, 159 aa, Streptomyces avidinii; identical to SEQ ID NO: 1
  REGION 1..159: note = 90% or more of the amino acid residues other than glycine in the amino acid sequence are D-amino acid residues

SEQ ID NO: 13 - protein, 127 aa, Gallus gallus
  REGION 1..127: note = 90% or more of the amino acid residues other than glycine in the core sequence are D-amino acid residues
RKCSLTGKWTNDLGSNMTIGAVNSRGEFTGTYITAVTATSNEIKESPLHGTQNTINKRTQPTFGFTVNWKFSESTTVFTGQCFIDRNGKEVLKTMWLLRSSVNDIGDDWKATRVGINIFTRLRTQKE

SEQ ID NO: 14 - protein, 128 aa, Gallus gallus; identical to SEQ ID NO: 2
  REGION 1..128: note = 90% or more of the amino acid residues other than glycine in the amino acid sequence are D-amino acid residues

SEQ ID NO: 15 - protein, 126 aa, Pleurotus cornucopiae
  REGION 1..126: note = 90% or more of the amino acid residues other than glycine in the core sequence are D-amino acid residues
VQSLLTGTWYNELGSTMNLTANKDGSLTGTYHSNVGEVPPTYHLSGRYNLQPPSGQGVTLGWAVSFENTSANVHSVSTWSGQYFSEPAEVILTQWLLSRSSEREDLWQSTHVGHDEFSKTKPTKEK

SEQ ID NO: 16 - protein, 143 aa, Pleurotus cornucopiae; identical to SEQ ID NO: 3
  REGION 1..143: note = 90% or more of the amino acid residues other than glycine in the amino acid sequence are D-amino acid residues

SEQ ID NO: 17 - protein, 124 aa, Pleurotus cornucopiae
  REGION 1..124: note = 90% or more of the amino acid residues other than glycine in the core sequence are D-amino acid residues
VQSSLTGTWYNELNSKMELTANKDGTLTGKYLSKVGDVYVPYPLSGRYNLQPPAGQGVALGWAVSWENSKIHSATTWSGQFFSESSPVILTQWLLSSSTARGDVWESTLVGNDSFTKTAPTEQQ

SEQ ID NO: 18 - protein, 141 aa, Pleurotus cornucopiae; identical to SEQ ID NO: 4
  REGION 1..141: note = 90% or more of the amino acid residues other than glycine in the amino acid sequence are D-amino acid residues

SEQ ID NO: 19 - protein, 115 aa, synthetic construct
  REGION 1..115: note = 90% or more of the amino acid residues other than glycine in the core sequence are D-amino acid residues
GTWYNQLGSTFIVTAGADGALTGTYEAAVGNAESRYVLTGRYDSAPATDGSGTALGWTVAWKNNYRNAHSAATWSGQYVGGAEARINTQWLLTSGTTEANAWKSTLVGHATFTKV

SEQ ID NO: 20 - protein, 121 aa, synthetic construct
  REGION 1..121: note = 90% or more of the amino acid residues other than glycine in the partial sequence are D-amino acid residues
AEAGITGTWYNQLGSTFIVTAGADGALTGTYEAAVGNAESRYVLTGRYDSAPATDGSGTALGWTVAWKNNYRNAHSAATWSGQYVGGAEARINTQWLLTSGTTEANAWKSTLVGHATFTKV

SEQ ID NO: 21 - protein, 159 aa, synthetic construct; identical to SEQ ID NO: 5
  REGION 1..159: note = 90% or more of the amino acid residues other than glycine in the amino acid sequence are D-amino acid residues

SEQ ID NO: 22 - protein, 115 aa, synthetic construct
  REGION 1..115: note = 90% or more of the amino acid residues other than glycine in the core sequence are D-amino acid residues
GTWYNQLGSTFIVTAGADGALTGTYESAVGNAESRYTLTGRYDSAPARDGSGTALGWTVAWKNNYRNAHSATTWSGQYVGGAEARINTQWTLTSGTTEANAWKSTLRGHDTFTKV

SEQ ID NO: 23 - protein, 121 aa, synthetic construct
  REGION 1..121: note = 90% or more of the amino acid residues other than glycine in the partial sequence are D-amino acid residues
AEAGITGTWYNQLGSTFIVTAGADGALTGTYESAVGNAESRYTLTGRYDSAPARDGSGTALGWTVAWKNNYRNAHSATTWSGQYVGGAEARINTQWTLTSGTTEANAWKSTLRGHDTFTKV

SEQ ID NO: 24 - protein, 159 aa, synthetic construct; identical to SEQ ID NO: 6
  REGION 1..159: note = 90% or more of the amino acid residues other than glycine in the amino acid sequence are D-amino acid residues

SEQ ID NO: 25 - protein, 114 aa, synthetic construct; identical to SEQ ID NO: 7
  REGION 1..114: note = 90% or more of the amino acid residues other than glycine in the amino acid sequence are D-amino acid residues

SEQ ID NO: 26 - protein, 107 aa, synthetic construct
  REGION 1..107: note = 90% or more of the amino acid residues other than glycine in the core sequence are D-amino acid residues
GTWYNQLGSTFIVTAGADGALTGTYESAVGNAESRYVLTGRYDSAPATDGSGTALGWTVAWKNNYRNAHSATTWSGQYVGGAEARINTQWLLTSKSTLVGDDTFTKV

SEQ ID NO: 27 - protein, 113 aa, synthetic construct
  REGION 1..113: note = 90% or more of the amino acid residues other than glycine in the partial sequence are D-amino acid residues
AEAGITGTWYNQLGSTFIVTAGADGALTGTYESAVGNAESRYVLTGRYDSAPATDGSGTALGWTVAWKNNYRNAHSATTWSGQYVGGAEARINTQWLLTSKSTLVGDDTFTKV

SEQ ID NO: 28 - protein, 113 aa, synthetic construct
  REGION 1..113: note = 90% or more of the amino acid residues other than glycine in the partial sequence are D-amino acid residues
GTWYNQLGSTFIVTAGADGALTGTYESAVGNAESRYVLTGRYDSAPATDGSGTALGWTVAWKNNYRNAHSATTWSGQYVGGAEARINTQWLLTSKSTLVGDDTFTKVKPSAAS

SEQ ID NO: 29 - protein, 119 aa, synthetic construct
  REGION 1..119: note = 90% or more of the amino acid residues other than glycine in the partial sequence are D-amino acid residues
AEAGITGTWYNQLGSTFIVTAGADGALTGTYESAVGNAESRYVLTGRYDSAPATDGSGTALGWTVAWKNNYRNAHSATTWSGQYVGGAEARINTQWLLTSKSTLVGDDTFTKVKPSAAS

SEQ ID NO: 30 - protein, 151 aa, synthetic construct; identical to SEQ ID NO: 8
  REGION 1..151: note = 90% or more of the amino acid residues other than glycine in the amino acid sequence are D-amino acid residues

SEQ ID NO: 31 - protein, 231 aa, synthetic construct
  REGION 1..231
EANAKKSTLVGHDTFTKVKPGTWYNQLGSTFIVTAGADGALTGTYESAVGNAESRYVLTGRYDSAPATDGSGTALGWTVAWKNNYRNAHSATTWSGQYVGGAEARINTQWLLTSGTGSGTALGWTVAWKNNYRNAHSATTWSGQYVGGAEARINTQWLLTSGTTEANAWKSTLVGHDTFTKVGTWYNQLGSTFIVTAGADGALTGTYESAVGNAESRYVLTGRYDSAPATD

SEQ ID NO: 32 - protein, 253 aa, synthetic construct
  REGION 1..253: note = 90% or more of the amino acid residues other than glycine in the partial sequence are D-amino acid residues
EANAKKSTLVGHDTFTKVKPSAASAEAGITGTWYNQLGSTFIVTAGADGALTGTYESAVGNAESRYVLTGRYDSAPATDGSGTALGWTVAWKNNYRNAHSATTWSGQYVGGAEARINTQWLLTSGTGSGTALGWTVAWKNNYRNAHSATTWSGQYVGGAEARINTQWLLTSGTTEANAWKSTLVGHDTFTKVKPSAASAEVGITGTWYNQLGSTFIVTAGADGALTGTYESAVGNAESRYVLTGRYDSAPATD

SEQ ID NO: 33 - protein, 273 aa, synthetic construct; identical to SEQ ID NO: 9
  REGION 1..273